European Patent Application EP 4 717 271 A1, published April 1, 2026. Title: 用于血管修复的164.88度重组III型人源化胶原蛋白. Applicant: 山西锦波生物医药股份有限公司. Application CN. The sequence listing filed with the application follows.

SEQUENCE LISTING (3 sequences)

SEQ ID NO: 1 - protein, 30 aa, synthetic construct
GERGAPGFRGPAGPNGIPGEKGPAGERGAP

SEQ ID NO: 2 - protein, 10 aa, synthetic construct
GPPGPCCGGG

SEQ ID NO: 3 - protein, 480 aa, synthetic construct
GERGAPGFRGPAGPNGIPGEKGPAGERGAPGERGAPGFRGPAGPNGIPGEKGPAGERGAPGERGAPGFRGPAGPNGIPGEKGPAGERGAPGERGAPGFRGPAGPNGIPGEKGPAGERGAPGERGAPGFRGPAGPNGIPGEKGPAGERGAPGERGAPGFRGPAGPNGIPGEKGPAGERGAPGERGAPGFRGPAGPNGIPGEKGPAGERGAPGERGAPGFRGPAGPNGIPGEKGPAGERGAPGERGAPGFRGPAGPNGIPGEKGPAGERGAPGERGAPGFRGPAGPNGIPGEKGPAGERGAPGERGAPGFRGPAGPNGIPGEKGPAGERGAPGERGAPGFRGPAGPNGIPGEKGPAGERGAPGERGAPGFRGPAGPNGIPGEKGPAGERGAPGERGAPGFRGPAGPNGIPGEKGPAGERGAPGERGAPGFRGPAGPNGIPGEKGPAGERGAPGERGAPGFRGPAGPNGIPGEKGPAGERGAP